European Patent Specification EP 3 712 131 B1, published February 1, 2023. Title: Neurotensin receptor ligands. Applicant: 3B Pharmaceuticals GmbH. The sequence listing filed with the application follows.

SEQUENCE LISTING (3 sequences)

SEQ ID NO: 1 - protein, 13 aa, Homo sapiens
  PEPTIDE (1)..(13): Neurotensin
ELYENKPRRPYIL

SEQ ID NO: 2 - protein, 8 aa, Homo sapiens
  MISC_FEATURE (1)..(8): Eight C-terminal amino acids of neurotensin
KPRRPYIL

SEQ ID NO: 3 - protein, 6 aa, Homo sapiens
  MISC_FEATURE (1)..(6): Six C-terminal amino acids of neurotensin
RRPYIL